European Patent Specification EP 4 423 111 B1, published December 4, 2024. Title: Peptides and compositions for use in cosmetics. Applicant: LIPOTRUE, S.L. The sequence listing filed with the application follows.

SEQUENCE LISTING (7 sequences)

SEQ ID NO: 1 - protein, 6 aa, Takifugu rubripes
  REGION 1..6: note = Peptide derived from the sequence of Nucleolar complex protein 2 homolog of the puffer fish Takifugu rubripes (Uniprot reference number: H2TGB2, amino acids 88 to 93).; note (original language) = Peptido derivado de la secuencia del homologo de la proteina 2 del complejo nucleolar del pez globo Takifugu rubripes (numero de referencia de Uniprot: H2TGB2, aminoacidos 88 a 93).
RWQKNQ

SEQ ID NO: 2 - protein, 6 aa, Takifugu rubripes
  REGION 1..6: note = Peptide derived from the sequence of Disabled homolog 2-interacting protein-like isoform X2 (Synaptic Ras-GTPase activating domain) (NCBI Reference Sequence: XP_003976523.1, amino acids 64 to 68).; note (original language) = Peptido derivado de la secuencia de la isoforma X2 similar a la proteina que interactua con el homologo desactivado 2 (dominio activador de Ras-GTPasa sinaptica) (Secuencia de referencia NCBI: XP_003976523.1, aminoacidos 64 a 68).
KRRYYC

SEQ ID NO: 3 - protein, 5 aa, Takifugu rubripes
  REGION 1..5: note = Peptide derived from a genome sequence predicted as calcium-independent phospholipase A2-gamma-like isoform X2 (NCBI Reference Sequence: XP_011605802.2, amino acids 7 to 11); note (original language) = Peptido derivado de una secuencia genomica predicha como isoforma X2 similar a la fosfolipasa A2 gamma independiente de calcio (Secuencia de referencia NCBI: XP_011605802.2, aminoacidos 7 a 11)
KHRSY

SEQ ID NO: 4 - protein, 5 aa, synthetic construct
  REGION 1..5: note = Artificially synthesized sequence; note (original language) = Secuencia sintetizada artificialmente
KDRVY

SEQ ID NO: 5 - protein, 6 aa, synthetic construct
  REGION 1..6: note = Artificially synthesized sequence; note (original language) = Secuencia sintetizada artificialmente
IEPYYV

SEQ ID NO: 6 - protein, 6 aa, synthetic construct
  REGION 1..6: note = Artificially synthesized sequence; note (original language) = Secuencia sintetizada artificialmente
KKHFWA

SEQ ID NO: 7 - skipped